European Patent Specification EP 3 740 590 B1, published April 24, 2024. Title: KITS AND METHODS FOR DIAGNOSING LUNG CANCER. Applicant: NUCLEIX LTD. The sequence listing filed with the application follows.

SEQUENCE LISTING (91 sequences)

SEQ ID NO: 1 - DNA, 85 bp, Homo sapiens
agtagcgcccactgagcggtttttcagttgctgcaccgttcttagcgcccaacggaacgtttcccgtacgcggagtccataagtt

SEQ ID NO: 2 - DNA, 69 bp, Homo sapiens
cggtcccgcagcgcccgccacacacccgcgccagaggtccagcgcatgtgcagtgaaatggcctagccc

SEQ ID NO: 3 - DNA, 72 bp, Homo sapiens
cggatagcgcggcgggcgacagccccccggataaccccgccgagggaggggcgcttgtaaaaccgagcggcg

SEQ ID NO: 4 - DNA, 60 bp, Homo sapiens
tcctccttgccttctttcgccgaaagggggcgcgctcctcccaggctgcgctggtaccta

SEQ ID NO: 5 - DNA, 78 bp, Homo sapiens
aggacccgctccgcaaagcgcccaccctcgagggaggaaagccgagctgcgcctccgcgcaaggccagggagtgtggc

SEQ ID NO: 6 - DNA, 73 bp, Homo sapiens
aggccgcgagcgcggcgcgatcagtagcgcccactaacagttcgttctgcacggcggagcgcgagaccgcgga

SEQ ID NO: 7 - DNA, 60 bp, Homo sapiens
agactaacttttctcttgtacagaatcatcaggctaaatttttggcattatttcagtcct

SEQ ID NO: 8 - DNA, 20 bp, Artificial Sequence
  Primer
tgcattctctcaggagctgg

SEQ ID NO: 9 - DNA, 19 bp, Artificial Sequence
  Primer
gagccaagctcggtctccg

SEQ ID NO: 10 - DNA, 21 bp, Artificial Sequence
  Primer
cagcaacgcttttgccagtag

SEQ ID NO: 11 - DNA, 20 bp, Artificial Sequence
  Primer
tctaatgcggagctggcggt

SEQ ID NO: 12 - DNA, 21 bp, Artificial Sequence
  Primer
cccactgagcggtttttcagt

SEQ ID NO: 13 - DNA, 20 bp, Artificial Sequence
  Primer
cgtttcccgtacgcggagtc

SEQ ID NO: 14 - DNA, 20 bp, Artificial Sequence
  Primer
gttttaatgtgttgtgacag

SEQ ID NO: 15 - DNA, 20 bp, Artificial Sequence
  Primer
gtgctgctagaaagaaactg

SEQ ID NO: 16 - DNA, 21 bp, Artificial Sequence
  Primer
gggtttaggaagttcctagga

SEQ ID NO: 17 - DNA, 20 bp, Artificial Sequence
  Primer
tactagttggcacagaggct

SEQ ID NO: 18 - DNA, 20 bp, Artificial Sequence
  Primer
cggtgccagaaccgagaaag

SEQ ID NO: 19 - DNA, 20 bp, Artificial Sequence
  Primer
accgttctgcaccgtaaaac

SEQ ID NO: 20 - DNA, 20 bp, Artificial Sequence
  Primer
cggaatagggtttgcaaatc

SEQ ID NO: 21 - DNA, 20 bp, Artificial Sequence
  Primer
aggagatgctgcttgttcgg

SEQ ID NO: 22 - DNA, 20 bp, Artificial Sequence
  Primer
gttgaagcttttaatacatg

SEQ ID NO: 23 - DNA, 19 bp, Artificial Sequence
  Primer
acagctcacggtcccgcag

SEQ ID NO: 24 - DNA, 17 bp, Artificial Sequence
  Primer
gcccgccacacacccgc

SEQ ID NO: 25 - DNA, 21 bp, Artificial Sequence
  Primer
cttgagatgaggttcccaagc

SEQ ID NO: 26 - DNA, 21 bp, Artificial Sequence
  Primer
agatgagtagcgagccttgtc

SEQ ID NO: 27 - DNA, 21 bp, Artificial Sequence
  Primer
cgtgctttgccgatcgaattc

SEQ ID NO: 28 - DNA, 20 bp, Artificial Sequence
  Primer
ttcctgctcgagtccactcg

SEQ ID NO: 29 - DNA, 21 bp, Artificial Sequence
  Primer
cgggtgtatcttcctgctcga

SEQ ID NO: 30 - DNA, 20 bp, Artificial Sequence
  Primer
cgagccttgacggagggaga

SEQ ID NO: 31 - DNA, 20 bp, Artificial Sequence
  Primer
cggagggagaatggaaagat

SEQ ID NO: 32 - DNA, 20 bp, Artificial Sequence
  Primer
tttcctccgccaccgagtag

SEQ ID NO: 33 - DNA, 21 bp, Artificial Sequence
  Primer
gaagtttaagtttccaggtcc

SEQ ID NO: 34 - DNA, 21 bp, Artificial Sequence
  Primer
atttgcgaagtttaagtttcc

SEQ ID NO: 35 - DNA, 20 bp, Artificial Sequence
  Primer
agcagccagggatcggatag

SEQ ID NO: 36 - DNA, 20 bp, Artificial Sequence
  Primer
tcggcagccgccctggtagc

SEQ ID NO: 37 - DNA, 20 bp, Artificial Sequence
  Primer
ccccatttgcgaagtttaag

SEQ ID NO: 38 - DNA, 20 bp, Artificial Sequence
  Primer
ggcagtctaatccttaattt

SEQ ID NO: 39 - DNA, 20 bp, Artificial Sequence
  Primer
attttaataatcaggataaa

SEQ ID NO: 40 - DNA, 21 bp, Artificial Sequence
  Primer
atgttcgagtcggtcgtaacg

SEQ ID NO: 41 - DNA, 23 bp, Artificial Sequence
  Primer
gtacacaaacgaatactagctaa

SEQ ID NO: 42 - DNA, 21 bp, Artificial Sequence
  Primer
ctaggcagtctaatccttaat

SEQ ID NO: 43 - DNA, 21 bp, Artificial Sequence
  Primer
atactagctaaggccgatgat

SEQ ID NO: 44 - DNA, 21 bp, Artificial Sequence
  Primer
ctctctgctgtagcgacgcca

SEQ ID NO: 45 - DNA, 21 bp, Artificial Sequence
  Primer
gctttccgccgggtaaattag

SEQ ID NO: 46 - DNA, 22 bp, Artificial Sequence
  Primer
tttggttatagtggtgtggtct

SEQ ID NO: 47 - DNA, 21 bp, Artificial Sequence
  Primer
ccaccccatcttcgcagttct

SEQ ID NO: 48 - DNA, 20 bp, Artificial Sequence
  Primer
tcctccttgccttctttcgc

SEQ ID NO: 49 - DNA, 22 bp, Artificial Sequence
  Primer
atagtggtgtggtctctgcctc

SEQ ID NO: 50 - DNA, 20 bp, Artificial Sequence
  Primer
gttttgttactgtctgtcct

SEQ ID NO: 51 - DNA, 21 bp, Artificial Sequence
  Primer
tcctgccaggtgtctacatgt

SEQ ID NO: 52 - DNA, 22 bp, Artificial Sequence
  Primer
actgtctgtcctgcaggaaccc

SEQ ID NO: 53 - DNA, 21 bp, Artificial Sequence
  Primer
tgaaggcaggataggtaccag

SEQ ID NO: 54 - DNA, 22 bp, Artificial Sequence
  Primer
tcaaactattatttcccacgtt

SEQ ID NO: 55 - DNA, 20 bp, Artificial Sequence
  Primer
acatgtttccattaagatgc

SEQ ID NO: 56 - DNA, 21 bp, Artificial Sequence
  Primer
cctgacgttcctggaatatgc

SEQ ID NO: 57 - DNA, 21 bp, Artificial Sequence
  Primer
gcaatgacttcttttaggaca

SEQ ID NO: 58 - DNA, 20 bp, Artificial Sequence
  Primer
tgaaagcagcattaaccgtg

SEQ ID NO: 59 - DNA, 19 bp, Artificial Sequence
  Primer
aggacccgctccgcaaagc

SEQ ID NO: 60 - DNA, 20 bp, Artificial Sequence
  Primer
accctcgagggaggaaagcc

SEQ ID NO: 61 - DNA, 21 bp, Artificial Sequence
  Primer
aacccgttactttccaaggac

SEQ ID NO: 62 - DNA, 19 bp, Artificial Sequence
  Primer
gccacactccctggccttg

SEQ ID NO: 63 - DNA, 19 bp, Artificial Sequence
  Primer
gcggggctcgagccacact

SEQ ID NO: 64 - DNA, 19 bp, Artificial Sequence
  Primer
cctccgcactgggaggctg

SEQ ID NO: 65 - DNA, 19 bp, Artificial Sequence
  Primer
tcgcagccgaggcaggtct

SEQ ID NO: 66 - DNA, 22 bp, Artificial Sequence
  Primer
cccgacagtgtcattgattaac

SEQ ID NO: 67 - DNA, 20 bp, Artificial Sequence
  Primer
cctccgcagctgggaggctg

SEQ ID NO: 68 - DNA, 20 bp, Artificial Sequence
  Primer
ctcggggactgctactttgc

SEQ ID NO: 69 - DNA, 20 bp, Artificial Sequence
  Primer
ggtcaagtgtcacgtcctcc

SEQ ID NO: 70 - DNA, 23 bp, Artificial Sequence
  Primer
atattcctgtaatgtatttaaat

SEQ ID NO: 71 - DNA, 19 bp, Artificial Sequence
  Primer
tacgcggggccgtgtgaat

SEQ ID NO: 72 - DNA, 20 bp, Artificial Sequence
  Primer
ggtcaagtgtcacgtcctcc

SEQ ID NO: 73 - DNA, 20 bp, Artificial Sequence
  Primer
aagtgtcacgtcctccgcaa

SEQ ID NO: 74 - DNA, 20 bp, Artificial Sequence
  Primer
gcgaggacgcaaacaccatt

SEQ ID NO: 75 - DNA, 20 bp, Artificial Sequence
  Primer
cctaaaggaccctaccaagc

SEQ ID NO: 76 - DNA, 21 bp, Artificial Sequence
  Primer
gtgcctgaactcttcctcctt

SEQ ID NO: 77 - DNA, 19 bp, Artificial Sequence
  Primer
ttccgtgggtccgcggtct

SEQ ID NO: 78 - DNA, 21 bp, Artificial Sequence
  Primer
atcagaaagaccattaggatc

SEQ ID NO: 79 - DNA, 21 bp, Artificial Sequence
  Primer
ccgaagggaaagaaaaatcag

SEQ ID NO: 80 - DNA, 23 bp, Artificial Sequence
  Primer
agcaaggtgaagactaacttttc

SEQ ID NO: 81 - DNA, 23 bp, Artificial Sequence
  Primer
cttgtacagaatcatcaggctaa

SEQ ID NO: 82 - DNA, 25 bp, Artificial Sequence
  Primer
gtccttggagacatctgagagattc

SEQ ID NO: 83 - DNA, 20 bp, Artificial Sequence
  Primer
gacatctgagagattccggg

SEQ ID NO: 84 - DNA, 22 bp, Artificial Sequence
  Primer
caaagaaagcaaggtgaagact

SEQ ID NO: 85 - DNA, 24 bp, Artificial Sequence
  Primer
cagtccttggagacatctgagaga

SEQ ID NO: 86 - DNA, 23 bp, Artificial Sequence
  Primer
tgaagtgaactattccttaggtg

SEQ ID NO: 87 - DNA, 23 bp, Artificial Sequence
  Primer
gtctccaaggactgaaataatgc

SEQ ID NO: 88 - DNA, 28 bp, Artificial Sequence
  Primer
gagtagcaaaaaatagctgaagtgaact

SEQ ID NO: 89 - DNA, 23 bp, Artificial Sequence
  Primer
tgacaaccaatgagtagcaaaaa

SEQ ID NO: 90 - DNA, 20 bp, Artificial Sequence
  Primer
gttgtcagtgtggccagaga

SEQ ID NO: 91 - DNA, 21 bp, Artificial Sequence
  Primer
tgttgtcagtgtggccagaga